European Patent Specification EP 3 252 162 B1, published March 1, 2023. Title: Method For Conducting Site-Specific Modification on Entire Plan Via Gene Transient Expression. Applicant: Institute of Genetics and Developmental Biology, Chinese Academy of Sciences. Application EP16742765.7. The sequence listing filed with the application follows.

SEQUENCE LISTING (5 sequences)

SEQ ID NO: 1 - DNA, 883 bp, Artificial
  pZmU3-gRNA-C1
gaattccatctaagtatcttggtaaagcatggattaatttggatgcccacttcaggtctatgcagctccggtgccttgtgattgtgagttgtgaccgatgctcatgctattctgcatttctgcgatgtatgtagctagtagatcttcaaaactaacaccgcatgccatcatcatccactgcttgattttagtctcaccgctggccaaaaatgtgatgatgccagaaacctcaactaccttgaatcaacacgggcccaacagtgtgatgacgacagaaacaaaaaaaaatgagccaatagttcagaaggaggcactatgcagaaactacatttctgaaggtgactaaaaggtgagcgtagagtgtaattactagtagtttagccaccattacccaaatgctttcgagcttgtattaagatttcctaagctgagcatcatcactgatctgcaggccaccctcgcttcgctgccaagatcaacagcaaccatgtggcggcaacatccagcattgcacatgggctaaagattgagctttgtgcctcgtctagggatcagctgaggttatcagtctttcctttttttcatccaggtgaggcatcaagctactactgcctcgattggctggacccgaagcccacatgtaggataccagaatgggccgacccaggacgcagtatgttggccagtcccaccggttagtgccatctcggttgctcacatgcgtagaagccagcttaaaaatttagctttggtgactcacagcagtcggcggcgtggtcgagctgttttagagctagaaatagcaagttaaaataaggctagtccgttatcaacttgaaaaagtggcaccgagtcggtgctttttttggtaccggatcctacg

SEQ ID NO: 2 - DNA, 4206 bp, Artificial
  Cas9 sequence in pJIT163-Ubi-Cas9
atggcccctaagaagaagagaaaggtcggtattcacggcgttcctgcggcgatggacaagaagtatagtattggtctggacattgggacgaattccgttggctgggccgtgatcaccgatgagtacaaggtcccttccaagaagtttaaggttctggggaacaccgatcggcacagcatcaagaagaatctcattggagccctcctgttcgactcaggcgagaccgccgaagcaacaaggctcaagagaaccgcaaggagacggtatacaagaaggaagaataggatctgctacctgcaggagattttcagcaacgaaatggcgaaggtggacgattcgttctttcatagattggaggagagtttcctcgtcgaggaagataagaagcacgagaggcatcctatctttggcaacattgtcgacgaggttgcctatcacgaaaagtaccccacaatctatcatctgcggaagaagcttgtggactcgactgataaggcggaccttagattgatctacctcgctctggcacacatgattaagttcaggggccattttctgatcgagggggatcttaacccggacaatagcgatgtggacaagttgttcatccagctcgtccaaacctacaatcagctctttgaggaaaacccaattaatgcttcaggcgtcgacgccaaggcgatcctgtctgcacgcctttcaaagtctcgccggcttgagaacttgatcgctcaactcccgggcgaaaagaagaacggcttgttcgggaatctcattgcactttcgttggggctcacaccaaacttcaagagtaattttgatctcgctgaggacgcaaagctgcagctttccaaggacacttatgacgatgacctggataaccttttggcccaaatcggcgatcagtacgcggacttgttcctcgccgcgaagaatttgtcggacgcgatcctcctgagtgatattctccgcgtgaacaccgagattacaaaggccccgctctcggcgagtatgatcaagcgctatgacgagcaccatcaggatctgacccttttgaaggctttggtccggcagcaactcccagagaagtacaaggaaatcttctttgatcaatccaagaacggctacgctggttatattgacggcggggcatcgcaggaggaattctacaagtttatcaagccaattctggagaagatggatggcacagaggaactcctggtgaagctcaatagggaggaccttttgcggaagcaaagaactttcgataacggcagcatccctcaccagattcatctcggggagctgcacgccatcctgagaaggcaggaagacttctacccctttcttaaggataaccgggagaagatcgaaaagattctgacgttcagaattccgtactatgtcggaccactcgcccggggtaattccagatttgcgtggatgaccagaaagagcgaggaaaccatcacaccttggaacttcgaggaagtggtcgataagggcgcttccgcacagagcttcattgagcgcatgacaaattttgacaagaacctgcctaatgagaaggtccttcccaagcattccctcctgtacgagtatttcactgtttataacgaactcacgaaggtgaagtatgtgaccgagggaatgcgcaagcccgccttcctgagcggcgagcaaaagaaggcgatcgtggaccttttgtttaagaccaatcggaaggtcacagttaagcagctcaaggaggactacttcaagaagattgaatgcttcgattccgttgagatcagcggcgtggaagacaggtttaacgcgtcactggggacttaccacgatctcctgaagatcattaaggataaggacttcttggacaacgaggaaaatgaggatatcctcgaagacattgtcctgactcttacgttgtttgaggatagggaaatgatcgaggaacgcttgaagacgtatgcccatctcttcgatgacaaggttatgaagcagctcaagagaagaagatacaccggatggggaaggctgtcccgcaagcttatcaatggcattagagacaagcaatcagggaagacaatccttgactttttgaagtctgatggcttcgcgaacaggaattttatgcagctgattcacgatgactcacttactttcaaggaggatatccagaaggctcaagtgtcgggacaaggtgacagtctgcacgagcatatcgccaaccttgcgggatctcctgcaatcaagaagggtattctgcagacagtcaaggttgtggatgagcttgtgaaggtcatgggacggcataagcccgagaacatcgttattgagatggccagagaaaatcagaccacacaaaagggtcagaagaactcgagggagcgcatgaagcgcatcgaggaaggcattaaggagctggggagtcagatccttaaggagcacccggtggaaaacacgcagttgcaaaatgagaagctctatctgtactatctgcaaaatggcagggatatgtatgtggaccaggagttggatattaaccgcctctcggattacgacgtcgatcatatcgttcctcagtccttccttaaggatgacagcattgacaataaggttctcaccaggtccgacaagaaccgcgggaagtccgataatgtgcccagcgaggaagtcgttaagaagatgaagaactactggaggcaacttttgaatgccaagttgatcacacagaggaagtttgataacctcactaaggccgagcgcggaggtctcagcgaactggacaaggcgggcttcattaagcggcaactggttgagactagacagatcacgaagcacgtggcgcagattctcgattcacgcatgaacacgaagtacgatgagaatgacaagctgatccgggaagtgaaggtcatcaccttgaagtcaaagctcgtttctgacttcaggaaggatttccaattttataaggtgcgcgagatcaacaattatcaccatgctcatgacgcatacctcaacgctgtggtcggaacagcattgattaagaagtacccgaagctcgagtccgaattcgtgtacggtgactataaggtttacgatgtgcgcaagatgatcgccaagtcagagcaggaaattggcaaggccactgcgaagtatttcttttactctaacattatgaatttctttaagactgagatcacgctggctaatggcgaaatccggaagagaccacttattgagaccaacggcgagacaggggaaatcgtgtgggacaaggggagggatttcgccacagtccgcaaggttctctctatgcctcaagtgaatattgtcaagaagactgaagtccagacgggcgggttctcaaaggaatctattctgcccaagcggaactcggataagcttatcgccagaaagaaggactgggacccgaagaagtatggaggtttcgactcaccaacggtggcttactctgtcctggttgtggcaaaggtggagaagggaaagtcaaagaagctcaagtctgtcaaggagctcctgggtatcaccattatggagaggtccagcttcgaaaagaatccgatcgattttctcgaggcgaagggatataaggaagtgaagaaggacctgatcattaagcttccaaagtacagtcttttcgagttggaaaacggcaggaagcgcatgttggcttccgcaggagagctccagaagggtaacgagcttgctttgccgtccaagtatgtgaacttcctctatctggcatcccactacgagaagctcaagggcagcccagaggataacgaacagaagcaactgtttgtggagcaacacaagcattatcttgacgagatcattgaacagatttcggagttcagtaagcgcgtcatcctcgccgacgcgaatttggataaggttctctcagcctacaacaagcaccgggacaagcctatcagagagcaggcggaaaatatcattcatctcttcaccctgacaaaccttggggctcccgctgcattcaagtattttgacactacgattgatcggaagagatacacttctacgaaggaggtgctggatgcaacccttatccaccaatcgattactggcctctacgagacgcggatcgacttgagtcagctcgggggggataagagaccagcggcaaccaagaaggcaggacaagcgaagaagaagaagtag

SEQ ID NO: 3 - DNA, 544 bp, Artificial
  gRNA sequence of pBUE411-C1
agtaattcatccaggtctccaagttctaggattttcagaactgcaacttattttatcaaggaatctttaaacatacgaacagatcacttaaagttcttctgaagcaacttaaagttatcaggcatgcatggatcttggaggaatcagatgtgcagtcagggaccatagcacaagacaggcgtcttctactggtgctaccagcaaatgctggaagccgggaacactgggtacgttggaaaccacgtgatgtgaagaagtaagataaactgtaggagaaaagcatttcgtagtgggccatgaagcctttcaggacatgtattgcagtatgggccggcccattacgcaattggacgacaacaaagactagtattagtaccacctcggctatccacatagatcaaagctgatttaaaagagttgtgcagatgatccgtggcggtcggcggcgtggtcgagctgttttagagctagaaatagcaagttaaaataaggctagtccgttatcaacttgaaaaagtggcaccgagtcggtgctttttttttt

SEQ ID NO: 4 - DNA, 4272 bp, Artificial
  Cas9 sequence of pHSN411-C1
atggattacaaggaccacgacggggattacaaggaccacgacattgattacaaggatgatgatgacaagatggctccgaagaagaagaggaaggttggcatccacggggtgccagctgctgacaagaagtactcgatcggcctcgatattgggactaactctgttggctgggccgtgatcaccgacgagtacaaggtgccctcaaagaagttcaaggtcctgggcaacaccgatcggcattccatcaagaagaatctcattggcgctctcctgttcgacagcggcgagacggctgaggctacgcggctcaagcgcaccgcccgcaggcggtacacgcgcaggaagaatcgcatctgctacctgcaggagattttctccaacgagatggcgaaggttgacgattctttcttccacaggctggaggagtcattcctcgtggaggaggataagaagcacgagcggcatccaatcttcggcaacattgtcgacgaggttgcctaccacgagaagtaccctacgatctaccatctgcggaagaagctcgtggactccacagataaggcggacctccgcctgatctacctcgctctggcccacatgattaagttcaggggccatttcctgatcgagggggatctcaacccggacaatagcgatgttgacaagctgttcatccagctcgtgcagacgtacaaccagctcttcgaggagaaccccattaatgcgtcaggcgtcgacgcgaaggctatcctgtccgctaggctctcgaagtctcggcgcctcgagaacctgatcgcccagctgccgggcgagaagaagaacggcctgttcgggaatctcattgcgctcagcctggggctcacgcccaacttcaagtcgaatttcgatctcgctgaggacgccaagctgcagctctccaaggacacatacgacgatgacctggataacctcctggcccagatcggcgatcagtacgcggacctgttcctcgctgccaagaatctgtcggacgccatcctcctgtctgatattctcagggtgaacaccgagattacgaaggctccgctctcagcctccatgatcaagcgctacgacgagcaccatcaggatctgaccctcctgaaggcgctggtcaggcagcagctccccgagaagtacaaggagatcttcttcgatcagtcgaagaacggctacgctgggtacattgacggcggggcctctcaggaggagttctacaagttcatcaagccgattctggagaagatggacggcacggaggagctgctggtgaagctcaatcgcgaggacctcctgaggaagcagcggacattcgataacggcagcatcccacaccagattcatctcggggagctgcacgctatcctgaggaggcaggaggacttctaccctttcctcaaggataaccgcgagaagatcgagaagattctgactttcaggatcccgtactacgtcggcccactcgctaggggcaactcccgcttcgcttggatgacccgcaagtcagaggagacgatcacgccgtggaacttcgaggaggtggtcgacaagggcgctagcgctcagtcgttcatcgagaggatgacgaatttcgacaagaacctgccaaatgagaaggtgctccctaagcactcgctcctgtacgagtacttcacagtctacaacgagctgactaaggtgaagtatgtgaccgagggcatgaggaagccggctttcctgtctggggagcagaagaaggccatcgtggacctcctgttcaagaccaaccggaaggtcacggttaagcagctcaaggaggactacttcaagaagattgagtgcttcgattcggtcgagatctctggcgttgaggaccgcttcaacgcctccctggggacctaccacgatctcctgaagatcattaaggataaggacttcctggacaacgaggagaatgaggatatcctcgaggacattgtgctgacactcactctgttcgaggaccgggagatgatcgaggagcgcctgaagacttacgcccatctcttcgatgacaaggtcatgaagcagctcaagaggaggaggtacaccggctgggggaggctgagcaggaagctcatcaacggcattcgggacaagcagtccgggaagacgatcctcgacttcctgaagagcgatggcttcgcgaaccgcaatttcatgcagctgattcacgatgacagcctcacattcaaggaggatatccagaaggctcaggtgagcggccagggggactcgctgcacgagcatatcgcgaacctcgctggctcgccagctatcaagaaggggattctgcagaccgtgaaggttgtggacgagctggtgaaggtcatgggcaggcacaagcctgagaacatcgtcattgagatggcccgggagaatcagaccacgcagaagggccagaagaactcacgcgagaggatgaagaggatcgaggagggcattaaggagctggggtcccagatcctcaaggagcacccggtggagaacacgcagctgcagaatgagaagctctacctgtactacctccagaatggccgcgatatgtatgtggaccaggagctggatattaacaggctcagcgattacgacgtcgatcatatcgttccacagtcattcctgaaggatgactccattgacaacaaggtcctcaccaggtcggacaagaaccggggcaagtctgataatgttccttcagaggaggtcgttaagaagatgaagaactactggcgccagctcctgaatgccaagctgatcacgcagcggaagttcgataacctcacaaaggctgagaggggcgggctctctgagctggacaaggcgggcttcatcaagaggcagctggtcgagacacggcagatcactaagcacgttgcgcagattctcgactcacggatgaacactaagtacgatgagaatgacaagctgatccgcgaggtgaaggtcatcaccctgaagtcaaagctcgtctccgacttcaggaaggatttccagttctacaaggttcgggagatcaacaattaccaccatgcccatgacgcgtacctgaacgcggtggtcggcacagctctgatcaagaagtacccaaagctcgagagcgagttcgtgtacggggactacaaggtttacgatgtgaggaagatgatcgccaagtcggagcaggagattggcaaggctaccgccaagtacttcttctactctaacattatgaatttcttcaagacagagatcactctggccaatggcgagatccggaagcgccccctcatcgagacgaacggcgagacgggggagatcgtgtgggacaagggcagggatttcgcgaccgtcaggaaggttctctccatgccacaagtgaatatcgtcaagaagacagaggtccagactggcgggttctctaaggagtcaattctgcctaagcggaacagcgacaagctcatcgcccgcaagaaggactgggatccgaagaagtacggcgggttcgacagccccactgtggcctactcggtcctggttgtggcgaaggttgagaagggcaagtccaagaagctcaagagcgtgaaggagctgctggggatcacgattatggagcgctccagcttcgagaagaacccgatcgatttcctggaggcgaagggctacaaggaggtgaagaaggacctgatcattaagctccccaagtactcactcttcgagctggagaacggcaggaagcggatgctggcttccgctggcgagctgcagaaggggaacgagctggctctgccgtccaagtatgtgaacttcctctacctggcctcccactacgagaagctcaagggcagccccgaggacaacgagcagaagcagctgttcgtcgagcagcacaagcattacctcgacgagatcattgagcagatttccgagttctccaagcgcgtgatcctggccgacgcgaatctggataaggtcctctccgcgtacaacaagcaccgcgacaagccaatcagggagcaggctgagaatatcattcatctcttcaccctgacgaacctcggcgcccctgctgctttcaagtacttcgacacaactatcgatcgcaagaggtacacaagcactaaggaggtcctggacgcgaccctcatccaccagtcgattaccggcctctacgagacgcgcatcgacctgtctcagctcgggggcgacaagcggccagcggcgacgaagaaggcggggcaggcgaagaagaagaagtga

SEQ ID NO: 5 - DNA, 487 bp, Artificial
  partial gDNA sequence of pHSN401-C2
aagcttcgacttgccttccgcacaatacatcatttcttcttagctttttttcttcttcttcgttcatacagtttttttttgtttatcagcttacattttcttgaaccgtagctttcgttttcttctttttaactttccattcggagtttttgtatcttgtttcatagtttgtcccaggattagaatgattaggcatcgaaccttcaagaatttgattgaataaaacatcttcattcttaagatatgaagataatcttcaaaaggcccctgggaatctgaaagaagagaagcaggcccatttatatgggaaagaacaatagtatttcttatataggcccatttaagttgaaaacaatcttcaaaagtcccacatcgcttagataagaaaacgaagctgagtttatatacagctagagtcgaagtagtgattggtgaaatcggcggatatcgtgttttagagctagaaatagcaagttaaaataaggct